European Patent Specification EP 3 941 509 B1, published December 3, 2025. Title: Factor IX variants and uses thereof in therapy. Applicant: CSL Behring Lengnau AG. Application EP19163619.0. The sequence listing filed with the application follows.

SEQUENCE LISTING (23 sequences)

SEQ ID NO: 1 - protein, 415 aa, Homo sapiens
YNSGKLEEFVQGNLERECMEEKCSFEEAREVFENTERTTEFWKQYVDGDQCESNPCLNGGSCKDDINSYECWCPFGFEGKNCELDVTCNIKNGRCEQFCKNSADNKVVCSCTEGYRLAENQKSCEPAVPFPCGRVSVSQTSKLTRAETVFPDVDYVNSTEAETILDNITQSTQSFNDFTRVVGGEDAKPGQFPWQVVLNGKVDAFCGGSIVNEKWIVTAAHCVETGVKITVVAGEHNIEETEHTEQKRNVIRIIPHHNYNAAINKYNHDIALLELDEPLVLNSYVTPICIADKEYTNIFLKFGSGYVSGWGRVFHKGRSALVLQYLRVPLVDRATCLRSTKFTIYNNMFCAGFHEGGRDSCQGDSGGPHVTEVEGTSFLTGIISWGEECAMKGKYGIYTKVSRYVNWIKEKTKLT

SEQ ID NO: 2 - DNA, 1251 bp, Homo sapiens
atgtataattcaggtaaattggaagagtttgttcaagggaaccttgagagagaatgtatggaagaaaagtgtagttttgaagaagcacgagaagtttttgaaaacactgaaagaacaactgaattttggaagcagtatgttgatggagatcagtgtgagtccaatccatgtttaaatggcggcagttgcaaggatgacattaattcctatgaatgttggtgtccctttggatttgaaggaaagaactgtgaattagatgtaacatgtaacattaagaatggcagatgcgagcagttttgtaaaaatagtgctgataacaaggtggtttgctcctgtactgagggatatcgacttgcagaaaaccagaagtcctgtgaaccagcagtgccatttccatgtggaagagtttctgtttcacaaacttctaagctcacccgtgctgagactgtttttcctgatgtggactatgtaaattctactgaagctgaaaccattttggataacatcactcaaagcacccaatcatttaatgacttcactcgggttgttggtggagaagatgccaaaccaggtcaattcccttggcaggttgttttgaatggtaaagttgatgcattctgtggaggctctatcgttaatgaaaaatggattgtaactgctgcccactgtgttgaaactggtgttaaaattacagttgtcgcaggtgaacataatattgaggagacagaacatacagagcaaaagcgaaatgtgattcgaattattcctcaccacaactacaatgcagctattaataagtacaaccatgacattgcccttctggaactggacgaacccttagtgctaaacagctacgttacacctatttgcattgctgacaaggaatacacgaacatcttcctcaaatttggatctggctatgtaagtggctggggaagagtcttccacaaagggagatcagctttagttcttcagtaccttagagttccacttgttgaccgagccacatgtcttcgatctacaaagttcaccatctataacaacatgttctgtgctggcttccatgaaggaggtagagattcatgtcaaggagatagtgggggaccccatgttactgaagtggaagggaccagtttcttaactggaattattagctggggtgaagagtgtgcaatgaaaggcaaatatggaatatataccaaggtatcccggtatgtcaactggattaaggaaaaaacaaagctcacttaa

SEQ ID NO: 3 - protein, 461 aa, Homo sapiens
MQRVNMIMAESPGLITICLLGYLLSAECTVFLDHENANKILNRPKRYNSGKLEEFVQGNLERECMEEKCSFEEAREVFENTERTTEFWKQYVDGDQCESNPCLNGGSCKDDINSYECWCPFGFEGKNCELDVTCNIKNGRCEQFCKNSADNKVVCSCTEGYRLAENQKSCEPAVPFPCGRVSVSQTSKLTRAETVFPDVDYVNSTEAETILDNITQSTQSFNDFTRVVGGEDAKPGQFPWQVVLNGKVDAFCGGSIVNEKWIVTAAHCVETGVKITVVAGEHNIEETEHTEQKRNVIRIIPHHNYNAAINKYNHDIALLELDEPLVLNSYVTPICIADKEYTNIFLKFGSGYVSGWGRVFHKGRSALVLQYLRVPLVDRATCLRSTKFTIYNNMFCAGFHEGGRDSCQGDSGGPHVTEVEGTSFLTGIISWGEECAMKGKYGIYTKVSRYVNWIKEKTKLT

SEQ ID NO: 4 - DNA, 1386 bp, Homo sapiens
atgcagcgcgtgaacatgatcatggcagaatcaccaggcctcatcaccatctgccttttaggatatctactcagtgctgaatgtacagtttttcttgatcatgaaaacgccaacaaaattctgaatcggccaaagaggtataattcaggtaaattggaagagtttgttcaagggaaccttgagagagaatgtatggaagaaaagtgtagttttgaagaagcacgagaagtttttgaaaacactgaaagaacaactgaattttggaagcagtatgttgatggagatcagtgtgagtccaatccatgtttaaatggcggcagttgcaaggatgacattaattcctatgaatgttggtgtccctttggatttgaaggaaagaactgtgaattagatgtaacatgtaacattaagaatggcagatgcgagcagttttgtaaaaatagtgctgataacaaggtggtttgctcctgtactgagggatatcgacttgcagaaaaccagaagtcctgtgaaccagcagtgccatttccatgtggaagagtttctgtttcacaaacttctaagctcacccgtgctgagactgtttttcctgatgtggactatgtaaattctactgaagctgaaaccattttggataacatcactcaaagcacccaatcatttaatgacttcactcgggttgttggtggagaagatgccaaaccaggtcaattcccttggcaggttgttttgaatggtaaagttgatgcattctgtggaggctctatcgttaatgaaaaatggattgtaactgctgcccactgtgttgaaactggtgttaaaattacagttgtcgcaggtgaacataatattgaggagacagaacatacagagcaaaagcgaaatgtgattcgaattattcctcaccacaactacaatgcagctattaataagtacaaccatgacattgcccttctggaactggacgaacccttagtgctaaacagctacgttacacctatttgcattgctgacaaggaatacacgaacatcttcctcaaatttggatctggctatgtaagtggctggggaagagtcttccacaaagggagatcagctttagttcttcagtaccttagagttccacttgttgaccgagccacatgtcttcgatctacaaagttcaccatctataacaacatgttctgtgctggcttccatgaaggaggtagagattcatgtcaaggagatagtgggggaccccatgttactgaagtggaagggaccagtttcttaactggaattattagctggggtgaagagtgtgcaatgaaaggcaaatatggaatatataccaaggtatcccggtatgtcaactggattaaggaaaaaacaaagctcacttaa

SEQ ID NO: 5 - protein, 145 aa, Homo sapiens
YNSGKLEEFVQGNLERECMEEKCSFEEAREVFENTERTTEFWKQYVDGDQCESNPCLNGGSCKDDINSYECWCPFGFEGKNCELDVTCNIKNGRCEQFCKNSADNKVVCSCTEGYRLAENQKSCEPAVPFPCGRVSVSQTSKLTR

SEQ ID NO: 6 - protein, 235 aa, Homo sapiens
VVGGEDAKPGQFPWQVVLNGKVDAFCGGSIVNEKWIVTAAHCVETGVKITVVAGEHNIEETEHTEQKRNVIRIIPHHNYNAAINKYNHDIALLELDEPLVLNSYVTPICIADKEYTNIFLKFGSGYVSGWGRVFHKGRSALVLQYLRVPLVDRATCLRSTKFTIYNNMFCAGFHEGGRDSCQGDSGGPHVTEVEGTSFLTGIISWGEECAMKGKYGIYTKVSRYVNWIKEKTKLT

SEQ ID NO: 7 - protein, 415 aa, Homo sapiens
YNSGKLEEFVQGNLERECMEEKCSFEEAREVFENTERTTEFWKQYVDGDQCESNPCLNGGSCKDDINSYECWCPFGFEGKNCELDVTCNIKNGRCEQFCKNSADNKVVCSCTEGYRLAENQKSCEPAVPFPCGRVSVSQTSKLTRAEAVFPDVDYVNSTEAETILDNITQSTQSFNDFTRVVGGEDAKPGQFPWQVVLNGKVDAFCGGSIVNEKWIVTAAHCVETGVKITVVAGEHNIEETEHTEQKRNVIRIIPHHNYNAAINKYNHDIALLELDEPLVLNSYVTPICIADKEYTNIFLKFGSGYVSGWGRVFHKGRSALVLQYLRVPLVDRATCLRSTKFTIYNNMFCAGFHEGGRDSCQGDSGGPHVTEVEGTSFLTGIISWGEECAMKGKYGIYTKVSRYVNWIKEKTKLT

SEQ ID NO: 8 - protein, 18 aa, Artificial Sequence
  Linker
PVSQTSKLTRAETVFPDV

SEQ ID NO: 9 - protein, 585 aa, Homo sapiens [sequence omitted]

SEQ ID NO: 10 - protein, 1018 aa, Artificial Sequence
  FIX (wild-type) albumin fusion protein
YNSGKLEEFVQGNLERECMEEKCSFEEAREVFENTERTTEFWKQYVDGDQCESNPCLNGGSCKDDINSYECWCPFGFEGKNCELDVTCNIKNGRCEQFCKNSADNKVVCSCTEGYRLAENQKSCEPAVPFPCGRVSVSQTSKLTRAETVFPDVDYVNSTEAETILDNITQSTQSFNDFTRVVGGEDAKPGQFPWQVVLNGKVDAFCGGSIVNEKWIVTAAHCVETGVKITVVAGEHNIEETEHTEQKRNVIRIIPHHNYNAAINKYNHDIALLELDEPLVLNSYVTPICIADKEYTNIFLKFGSGYVSGWGRVFHKGRSALVLQYLRVPLVDRATCLRSTKFTIYNNMFCAGFHEGGRDSCQGDSGGPHVTEVEGTSFLTGIISWGEECAMKGKYGIYTKVSRYVNWIKEKTKLTPVSQTSKLTRAETVFPDVDAHKSEVAHRFKDLGEENFKALVLIAFAQYLQQCPFEDHVKLVNEVTEFAKTCVADESAENCDKSLHTLFGDKLCTVATLRETYGEMADCCAKQEPERNECFLQHKDDNPNLPRLVRPEVDVMCTAFHDNEETFLKKYLYEIARRHPYFYAPELLFFAKRYKAAFTECCQAADKAACLLPKLDELRDEGKASSAKQRLKCASLQKFGERAFKAWAVARLSQRFPKAEFAEVSKLVTDLTKVHTECCHGDLLECADDRADLAKYICENQDSISSKLKECCEKPLLEKSHCIAEVENDEMPADLPSLAADFVESKDVCKNYAEAKDVFLGMFLYEYARRHPDYSVVLLLRLAKTYETTLEKCCAAADPHECYAKVFDEFKPLVEEPQNLIKQNCELFEQLGEYKFQNALLVRYTKKVPQVSTPTLVEVSRNLGKVGSKCCKHPEAKRMPCAEDYLSVVLNQLCVLHEKTPVSDRVTKCCTESLVNRRPCFSALEVDETYVPKEFNAETFTFHADICTLSEKERQIKKQTALVELVKHKPKATKEQLKAVMDDFAAFVEKCCKADDKETCFAEEGKKLVAASQAALGL

SEQ ID NO: 11 - protein, 415 aa, Artificial Sequence
  FIX variant R338V/E410H
YNSGKLEEFVQGNLERECMEEKCSFEEAREVFENTERTTEFWKQYVDGDQCESNPCLNGGSCKDDINSYECWCPFGFEGKNCELDVTCNIKNGRCEQFCKNSADNKVVCSCTEGYRLAENQKSCEPAVPFPCGRVSVSQTSKLTRAETVFPDVDYVNSTEAETILDNITQSTQSFNDFTRVVGGEDAKPGQFPWQVVLNGKVDAFCGGSIVNEKWIVTAAHCVETGVKITVVAGEHNIEETEHTEQKRNVIRIIPHHNYNAAINKYNHDIALLELDEPLVLNSYVTPICIADKEYTNIFLKFGSGYVSGWGRVFHKGRSALVLQYLRVPLVDRATCLVSTKFTIYNNMFCAGFHEGGRDSCQGDSGGPHVTEVEGTSFLTGIISWGEECAMKGKYGIYTKVSRYVNWIKHKTKLT

SEQ ID NO: 12 - protein, 415 aa, Artificial Sequence
  FIX variant R338T/E410H
YNSGKLEEFVQGNLERECMEEKCSFEEAREVFENTERTTEFWKQYVDGDQCESNPCLNGGSCKDDINSYECWCPFGFEGKNCELDVTCNIKNGRCEQFCKNSADNKVVCSCTEGYRLAENQKSCEPAVPFPCGRVSVSQTSKLTRAETVFPDVDYVNSTEAETILDNITQSTQSFNDFTRVVGGEDAKPGQFPWQVVLNGKVDAFCGGSIVNEKWIVTAAHCVETGVKITVVAGEHNIEETEHTEQKRNVIRIIPHHNYNAAINKYNHDIALLELDEPLVLNSYVTPICIADKEYTNIFLKFGSGYVSGWGRVFHKGRSALVLQYLRVPLVDRATCLTSTKFTIYNNMFCAGFHEGGRDSCQGDSGGPHVTEVEGTSFLTGIISWGEECAMKGKYGIYTKVSRYVNWIKHKTKLT

SEQ ID NO: 13 - protein, 415 aa, Artificial Sequence
  FIX variant R338W/E410H
YNSGKLEEFVQGNLERECMEEKCSFEEAREVFENTERTTEFWKQYVDGDQCESNPCLNGGSCKDDINSYECWCPFGFEGKNCELDVTCNIKNGRCEQFCKNSADNKVVCSCTEGYRLAENQKSCEPAVPFPCGRVSVSQTSKLTRAETVFPDVDYVNSTEAETILDNITQSTQSFNDFTRVVGGEDAKPGQFPWQVVLNGKVDAFCGGSIVNEKWIVTAAHCVETGVKITVVAGEHNIEETEHTEQKRNVIRIIPHHNYNAAINKYNHDIALLELDEPLVLNSYVTPICIADKEYTNIFLKFGSGYVSGWGRVFHKGRSALVLQYLRVPLVDRATCLWSTKFTIYNNMFCAGFHEGGRDSCQGDSGGPHVTEVEGTSFLTGIISWGEECAMKGKYGIYTKVSRYVNWIKHKTKLT

SEQ ID NO: 14 - protein, 415 aa, Artificial Sequence
  FIX variant R338L/E410H
YNSGKLEEFVQGNLERECMEEKCSFEEAREVFENTERTTEFWKQYVDGDQCESNPCLNGGSCKDDINSYECWCPFGFEGKNCELDVTCNIKNGRCEQFCKNSADNKVVCSCTEGYRLAENQKSCEPAVPFPCGRVSVSQTSKLTRAETVFPDVDYVNSTEAETILDNITQSTQSFNDFTRVVGGEDAKPGQFPWQVVLNGKVDAFCGGSIVNEKWIVTAAHCVETGVKITVVAGEHNIEETEHTEQKRNVIRIIPHHNYNAAINKYNHDIALLELDEPLVLNSYVTPICIADKEYTNIFLKFGSGYVSGWGRVFHKGRSALVLQYLRVPLVDRATCLLSTKFTIYNNMFCAGFHEGGRDSCQGDSGGPHVTEVEGTSFLTGIISWGEECAMKGKYGIYTKVSRYVNWIKHKTKLT

SEQ ID NO: 15 - protein, 1018 aa, Artificial Sequence
  FIX variant R338V/E410H albumin fusion
YNSGKLEEFVQGNLERECMEEKCSFEEAREVFENTERTTEFWKQYVDGDQCESNPCLNGGSCKDDINSYECWCPFGFEGKNCELDVTCNIKNGRCEQFCKNSADNKVVCSCTEGYRLAENQKSCEPAVPFPCGRVSVSQTSKLTRAETVFPDVDYVNSTEAETILDNITQSTQSFNDFTRVVGGEDAKPGQFPWQVVLNGKVDAFCGGSIVNEKWIVTAAHCVETGVKITVVAGEHNIEETEHTEQKRNVIRIIPHHNYNAAINKYNHDIALLELDEPLVLNSYVTPICIADKEYTNIFLKFGSGYVSGWGRVFHKGRSALVLQYLRVPLVDRATCLVSTKFTIYNNMFCAGFHEGGRDSCQGDSGGPHVTEVEGTSFLTGIISWGEECAMKGKYGIYTKVSRYVNWIKHKTKLTPVSQTSKLTRAETVFPDVDAHKSEVAHRFKDLGEENFKALVLIAFAQYLQQCPFEDHVKLVNEVTEFAKTCVADESAENCDKSLHTLFGDKLCTVATLRETYGEMADCCAKQEPERNECFLQHKDDNPNLPRLVRPEVDVMCTAFHDNEETFLKKYLYEIARRHPYFYAPELLFFAKRYKAAFTECCQAADKAACLLPKLDELRDEGKASSAKQRLKCASLQKFGERAFKAWAVARLSQRFPKAEFAEVSKLVTDLTKVHTECCHGDLLECADDRADLAKYICENQDSISSKLKECCEKPLLEKSHCIAEVENDEMPADLPSLAADFVESKDVCKNYAEAKDVFLGMFLYEYARRHPDYSVVLLLRLAKTYETTLEKCCAAADPHECYAKVFDEFKPLVEEPQNLIKQNCELFEQLGEYKFQNALLVRYTKKVPQVSTPTLVEVSRNLGKVGSKCCKHPEAKRMPCAEDYLSVVLNQLCVLHEKTPVSDRVTKCCTESLVNRRPCFSALEVDETYVPKEFNAETFTFHADICTLSEKERQIKKQTALVELVKHKPKATKEQLKAVMDDFAAFVEKCCKADDKETCFAEEGKKLVAASQAALGL

SEQ ID NO: 16 - protein, 231 aa, Homo sapiens
EPKSCDKTHTCPPCPAPELLGGPSVFLFPPKPKDTLMISRTPEVTCVVVDVSHEDPEVKFNWYVDGVEVHNAKTKPREEQYNSTYRVVSVLTVLHQDWLNGKEYKCKVSNKALPAPIEKTISKAKGQPREPQVYTLPPSRDELTKNQVSLTCLVKGFYPSDIAVEWESNGQPENNYKTTPPVLDSDGSFFLYSKLTVDKSRWQQGNVFSCSVMHEALHNHYTQKSLSLSPG

SEQ ID NO: 17 - protein, 226 aa, Homo sapiens
DKTHTCPPCPAPELLGGPSVFLFPPKPKDTLMISRTPEVTCVVVDVSHEDPEVKFNWYVDGVEVHNAKTKPREEQYNSTYRVVSVLTVLHQDWLNGKEYKCKVSNKALPAPIEKTISKAKGQPREPQVYTLPPSRDELTKNQVSLTCLVKGFYPSDIAVEWESNGQPENNYKTTPPVLDSDGSFFLYSKLTVDKSRWQQGNVFSCSVMHEALHNHYTQKSLSLSPG

SEQ ID NO: 18 - protein, 10 aa, Artificial Sequence
  CTP sequence
SSSSKAPPPS

SEQ ID NO: 19 - protein, 32 aa, Artificial Sequence
  CTP sequence
DPRFQDSSSSKAPPPSLPSPSRLPGPSDTPIL

SEQ ID NO: 20 - protein, 28 aa, Artificial Sequence
  CTP sequence
SSSSKAPPPSLPSPSRLPGPSDTPILPQ

SEQ ID NO: 21 - protein, 78 aa, Artificial Sequence
  XTEN artificial sequence
GAPTSESATPESGPGSEPATSGSETPGTSESATPESGPGSEPATSGSETPGTSESATPESGPGTSTEPSEGSAPGASS

SEQ ID NO: 22 - protein, 42 aa, Artificial Sequence
  XTEN artificial sequence
GAPGSPAGSPTSTEEGTSESATPESGPGSEPATSGSETPASS

SEQ ID NO: 23 - protein, 7 aa, Artificial Sequence
  Linker
GGGGGGV